European Patent Application EP 4 435 111 A1, published September 25, 2024. Title: Digital Analyte Analysis. Applicant: Bio-Rad Laboratories, Inc. Application EP 11742907.6, filed February 11, 2011. The sequence listing filed with the application follows.

SEQUENCE LISTING (14 sequences)

SEQ ID NO: 1 - DNA, 27 bp, synthetic construct
  misc_feature 1..27: note = Synthetic oligonucleotide
  source 1..27: mol_type = other DNA
aatgctttttaacatccatataaagct

SEQ ID NO: 2 - DNA, 25 bp, synthetic construct
  misc_feature 1..25: note = Synthetic oligonucleotide
  source 1..25: mol_type = other DNA
ccttaatttaaggaatgtgagcacc

SEQ ID NO: 3 - DNA, 16 bp, synthetic construct
  misc_feature 1..16: note = Synthetic oligonucleotide
  source 1..16: mol_type = other DNA
cagggtttcagacaaa

SEQ ID NO: 4 - DNA, 27 bp, synthetic construct
  misc_feature 1..27: note = Synthetic oligonucleotide
  source 1..27: mol_type = other DNA
aatgctttttaacatccatataaagct

SEQ ID NO: 5 - DNA, 25 bp, synthetic construct
  misc_feature 1..25: note = Synthetic oligonucleotide
  source 1..25: mol_type = other DNA
ccttaatttaaggaatgtgagcacc

SEQ ID NO: 6 - DNA, 18 bp, synthetic construct
  misc_feature 1..18: note = Synthetic oligonucleotide
  source 1..18: mol_type = other DNA
tgattttgtctaaaaccc

SEQ ID NO: 7 - DNA, 24 bp, synthetic construct
  misc_feature 1..24: note = Synthetic oligonucleotide
  source 1..24: mol_type = other DNA
caacctactcttctcagacgtgta

SEQ ID NO: 8 - DNA, 23 bp, synthetic construct
  misc_feature 1..23: note = Synthetic oligonucleotide
  source 1..23: mol_type = other DNA
tcgaagtgatccagtgggtagtg

SEQ ID NO: 9 - DNA, 21 bp, synthetic construct
  misc_feature 1..21: note = Synthetic oligonucleotide
  source 1..21: mol_type = other DNA
caggagatgcccgcccagctc

SEQ ID NO: 10 - DNA, 25 bp, synthetic construct
  misc_feature 1..25: note = Synthetic oligonucleotide
  source 1..25: mol_type = other DNA
tgctgatgctttgggaagtatgtta

SEQ ID NO: 11 - DNA, 18 bp, synthetic construct
  misc_feature 1..18: note = Synthetic oligonucleotide
  source 1..18: mol_type = other DNA
catgagtggctatcatac

SEQ ID NO: 12 - DNA, 25 bp, synthetic construct
  misc_feature 1..25: note = Synthetic oligonucleotide
  source 1..25: mol_type = other DNA
tgtcaggaaaagatgctgagtgatt

SEQ ID NO: 13 - DNA, 17 bp, synthetic construct
  misc_feature 1..17: note = Synthetic oligonucleotide
  source 1..17: mol_type = other DNA
atgagtggctgtcatac

SEQ ID NO: 14 - DNA, 18 bp, synthetic construct
  misc_feature 1..18: note = Synthetic oligonucleotide
  source 1..18: mol_type = other DNA
catgagtggctgtcatac